European Patent Application EP 4 299 723 A1, published January 3, 2024. Title: A genetically modified cell and method for production thereof. Applicant: Showa Denko Materials Co., Ltd. National Cancer Center. The sequence listing filed with the application follows.

SEQUENCE LISTING (3 sequences)

SEQ ID NO: 1 - DNA, 1371 bp, Artificial Sequence
  CD8
atggccttaccagtgaccgccttgctcctgccgctggccttgctgctccacgccgccaggccgagccagttccgggtgtcgccgctggatcggacctggaacctgggcgagacagtggagctgaagtgccaggtgctgctgtccaacccgacgtcgggctgctcgtggctcttccagccgcgcggcgccgccgccagtcccaccttcctcctatacctctcccaaaacaagcccaaggcggccgaggggctggacacccagcggttctcgggcaagaggttgggggacaccttcgtcctcaccctgagcgacttccgccgagagaacgagggctactatttctgctcggccctgagcaactccatcatgtacttcagccacttcgtgccggtcttcctgccagcgaagcccaccacgacgccagcgccgcgaccaccaacaccggcgcccaccatcgcgtcgcagcccctgtccctgcgcccagaggcgtgccggccagcggcggggggcgcagtgcacacgagggggctggacttcgcctgtgatatctacatctgggcgcccttggccgggacttgtggggtccttctcctgtcactggttatcaccctttactgcaaccacaggaaccgaagacgtgtttgcaaatgtccccggcctgtggtcaaatcgggagacaagcccagcctttcggcgagatacgtctccggaagcggagccaccaacttcagcctgctgaagcaggccggtgacgtcgaggagaatcctggccccatgcggccgcggctgtggctcctcttggccgcgcagctgacagttctccatggcaactcagtcctccagcagacccctgcatacataaaggtgcaaaccaacaagatggtgatgctgtcctgcgaggctaaaatctccctcagtaacatgcgcatctactggctgagacagcgccaggcaccgagcagtgacagtcaccacgagttcctggccctctgggattccgcaaaagggactatccacggtgaagaggtggaacaggagaagatagctgtgtttcgggatgcaagccggttcattctcaatctcacaagcgtgaagccggaagacagtggcatctacttctgcatgatcgtcgggagccccgagctgaccttcgggaagggaactcagctgagtgtggttgatttccttcccaccactgcccagcccaccaagaagtccaccctcaagaagagagtgtgccggttacccaggccagagacccagaagggcctcaaggggaaggtatatcaggaacctttgtcccccaatgcctgcatggatactacagcaatactacaacctcacagaagctgcttaacccatggatcctga

SEQ ID NO: 2 - DNA, 705 bp, Artificial Sequence
  CD8A
atggccttaccagtgaccgccttgctcctgccgctggccttgctgctccacgccgccaggccgagccagttccgggtgtcgccgctggatcggacctggaacctgggcgagacagtggagctgaagtgccaggtgctgctgtccaacccgacgtcgggctgctcgtggctcttccagccgcgcggcgccgccgccagtcccaccttcctcctatacctctcccaaaacaagcccaaggcggccgaggggctggacacccagcggttctcgggcaagaggttgggggacaccttcgtcctcaccctgagcgacttccgccgagagaacgagggctactatttctgctcggccctgagcaactccatcatgtacttcagccacttcgtgccggtcttcctgccagcgaagcccaccacgacgccagcgccgcgaccaccaacaccggcgcccaccatcgcgtcgcagcccctgtccctgcgcccagaggcgtgccggccagcggcggggggcgcagtgcacacgagggggctggacttcgcctgtgatatctacatctgggcgcccttggccgggacttgtggggtccttctcctgtcactggttatcaccctttactgcaaccacaggaaccgaagacgtgtttgcaaatgtccccggcctgtggtcaaatcgggagacaagcccagcctttcggcgagatacgtc

SEQ ID NO: 3 - DNA, 597 bp, Artificial Sequence
  CD8B
atgcggccgcggctgtggctcctcttggccgcgcagctgacagttctccatggcaactcagtcctccagcagacccctgcatacataaaggtgcaaaccaacaagatggtgatgctgtcctgcgaggctaaaatctccctcagtaacatgcgcatctactggctgagacagcgccaggcaccgagcagtgacagtcaccacgagttcctggccctctgggattccgcaaaagggactatccacggtgaagaggtggaacaggagaagatagctgtgtttcgggatgcaagccggttcattctcaatctcacaagcgtgaagccggaagacagtggcatctacttctgcatgatcgtcgggagccccgagctgaccttcgggaagggaactcagctgagtgtggttgatttccttcccaccactgcccagcccaccaagaagtccaccctcaagaagagagtgtgccggttacccaggccagagacccagaagggcctcaaggggaaggtatatcaggaacctttgtcccccaatgcctgcatggatactacagcaatactacaacctcacagaagctgcttaacccatggatcctga